European Patent Application EP 4 549 558 A1, published May 7, 2025. Title: BACTERIA-TARGETING CAPSID PARTICLE, TREATMENT COMPOSITION, DISINFECTANT, FOOD, BACTERIA ELIMINATION METHOD, BACTERICIDAL METHOD, CORROSION PREVENTION METHOD, ANIMAL TREATMENT METHOD, GENE INTRODUCTION METHOD, BACTERIA FUNCTION ADDITION METHOD, METHOD FOR PRODUCING BACTERIA-TARGETING CAPSID PARTICLE, AND METHOD FOR PRODUCING NUCLEIC ACID FOR BACTERIA-TARGETING CAPSID PARTICLE. Applicant: JICHI MEDICAL UNIVERSITY. Application EP 23828679.3, filed June 26, 2023. The sequence listing filed with the application follows.

SEQUENCE LISTING (72 sequences)

SEQ ID NO: 1 - DNA, 40 bp, Escherichia coli
  source 1..40: mol_type = other DNA
taaactcaaggtccctaaattaatacgactcactataggg

SEQ ID NO: 2 - DNA, 40 bp, Escherichia coli
  source 1..40: mol_type = other DNA
ccacagggagaatatttaattaaataccggaacttctccg

SEQ ID NO: 3 - DNA, 40 bp, Escherichia coli
  source 1..40: mol_type = other DNA
cggagaagttccggtatttaattaaatattctccctgtgg

SEQ ID NO: 4 - DNA, 40 bp, Escherichia coli
  source 1..40: mol_type = other DNA
ctacacgtctttccttgtgatttaccaattactcgttctc

SEQ ID NO: 5 - DNA, 77 bp, Escherichia coli
  source 1..77: mol_type = other DNA
gagaacgagtaattggtaaatcacaaggaaagacgtgtagaaatcataccaacatggtcaaataaaacgaaaggctc

SEQ ID NO: 6 - DNA, 73 bp, Escherichia coli
  source 1..73: mol_type = other DNA
ccctatagtgagtcgtattaatttagggaccttgagtttactaaatactagtgactccagcgtaactggactg

SEQ ID NO: 7 - DNA, 20 bp, Escherichia coli
  source 1..20: mol_type = other DNA
ctttctctgtccttcctgtg

SEQ ID NO: 8 - DNA, 20 bp, Escherichia coli
  source 1..20: mol_type = other DNA
ctggaatatcgttagggttc

SEQ ID NO: 9 - DNA, 20 bp, Escherichia coli
  source 1..20: mol_type = other DNA
acaatatcgattccctgtgg

SEQ ID NO: 10 - DNA, 20 bp, Escherichia coli
  source 1..20: mol_type = other DNA
tcaagaatgtcatggtgagc

SEQ ID NO: 11 - DNA, 20 bp, Escherichia coli
  source 1..20: mol_type = other DNA
cttcatagcctctgatggtg

SEQ ID NO: 12 - DNA, 20 bp, Escherichia coli
  source 1..20: mol_type = other DNA
tttagcttccttagctcctg

SEQ ID NO: 13 - DNA, 74 bp, Escherichia coli
  source 1..74: mol_type = other DNA
cttagccagaataatcaagtcgttacacgacactaagtgatccacggatggactctcaaggaggtacaaggtgc

SEQ ID NO: 14 - DNA, 35 bp, Escherichia coli
  source 1..35: mol_type = other DNA
gctttcacttcctcaaaccagtcgttgatgcgtgc

SEQ ID NO: 15 - DNA, 35 bp, Escherichia coli
  source 1..35: mol_type = other DNA
tgattgcacgcatcaacgactggtttgaggaagtg

SEQ ID NO: 16 - DNA, 35 bp, Escherichia coli
  source 1..35: mol_type = other DNA
caactgctttgaaaccttgtcctctaggccagagc

SEQ ID NO: 17 - DNA, 35 bp, Escherichia coli
  source 1..35: mol_type = other DNA
gtttcgctctggcctagaggacaaggtttcaaagc

SEQ ID NO: 18 - DNA, 43 bp, Escherichia coli
  source 1..43: mol_type = other DNA
tcacttagtgtcgtgtaacgacttgattattctggctaagtcc

SEQ ID NO: 19 - DNA, 20 bp, Escherichia coli
  source 1..20: mol_type = other DNA
ccaagcctctcatcactacc

SEQ ID NO: 20 - DNA, 20 bp, Escherichia coli
  source 1..20: mol_type = other DNA
tgcttagcttcaaggtcacg

SEQ ID NO: 21 - DNA, 20 bp, Escherichia coli
  source 1..20: mol_type = other DNA
tatggtgtctcccaacagac

SEQ ID NO: 22 - DNA, 20 bp, Escherichia coli
  source 1..20: mol_type = other DNA
ccataagacgttggagaacc

SEQ ID NO: 23 - DNA, 20 bp, Escherichia coli
  source 1..20: mol_type = other DNA
ttacctgtggagaccgtagc

SEQ ID NO: 24 - DNA, 20 bp, Escherichia coli
  source 1..20: mol_type = other DNA
aacttgtggcggtctaacag

SEQ ID NO: 25 - DNA, 30 bp, Escherichia coli
  source 1..30: mol_type = other DNA
tagcggataactcaagggtatcgcaaggtg

SEQ ID NO: 26 - DNA, 30 bp, Escherichia coli
  source 1..30: mol_type = other DNA
tttctcccgcagttccacttagaagtctcc

SEQ ID NO: 27 - DNA, 30 bp, Escherichia coli
  source 1..30: mol_type = other DNA
tgaagtgtcacgaagaggcttatgctgctg

SEQ ID NO: 28 - DNA, 30 bp, Escherichia coli
  source 1..30: mol_type = other DNA
cgagccatttggccctgcttgataatatcc

SEQ ID NO: 29 - DNA, 30 bp, Escherichia coli
  source 1..30: mol_type = other DNA
tgtaccactggtaacatcctgactcagacc

SEQ ID NO: 30 - DNA, 30 bp, Escherichia coli
  source 1..30: mol_type = other DNA
ccaaagtcccaatgagaccacgactgttgc

SEQ ID NO: 31 - DNA, 30 bp, Escherichia coli
  source 1..30: mol_type = other DNA
cttccgtaaccgcttaggattccttagtgg

SEQ ID NO: 32 - DNA, 30 bp, Escherichia coli
  source 1..30: mol_type = other DNA
aagctgttgagtcaatgggtcgttcggtac

SEQ ID NO: 33 - DNA, 30 bp, Escherichia coli
  source 1..30: mol_type = other DNA
tttctatgctatggctgcacacgtcaaagc

SEQ ID NO: 34 - DNA, 30 bp, Escherichia coli
  source 1..30: mol_type = other DNA
ttcatcctcctcgtactcctcgacttcctc

SEQ ID NO: 35 - DNA, 35 bp, Escherichia coli
  source 1..35: mol_type = other DNA
aagccgtgtctttcgtagagtctgccattaagaag

SEQ ID NO: 36 - DNA, 35 bp, Escherichia coli
  source 1..35: mol_type = other DNA
tcatggtacttaacgtcctccagttcagcttccag

SEQ ID NO: 37 - DNA, 35 bp, Escherichia coli
  source 1..35: mol_type = other DNA
ctaaactggaagctgaactggaggacgttaagtac

SEQ ID NO: 38 - DNA, 35 bp, Escherichia coli
  source 1..35: mol_type = other DNA
ataaatcaccactcaatgaaagacgtaccgtaacc

SEQ ID NO: 39 - DNA, 70 bp, Staphylococcus aureus
  source 1..70: mol_type = other DNA
ggttacggtacgtctttcattgagtggtgatttatgtttaatcgcgactgtacgacgtagaaaagctagc

SEQ ID NO: 40 - DNA, 70 bp, Staphylococcus aureus
  source 1..70: mol_type = other DNA
ggttacggtacgtctttcattgagtggtgatttataaaggagaaagagatgacgttagaacgcgtgaaac

SEQ ID NO: 41 - DNA, 70 bp, Staphylococcus aureus
  source 1..70: mol_type = other DNA
ggttacggtacgtctttcattgagtggtgatttatcctcaacacaaaaaccaactcacacagcaacgttc

SEQ ID NO: 42 - DNA, 70 bp, Staphylococcus aureus
  source 1..70: mol_type = other DNA
ggttacggtacgtctttcattgagtggtgatttatttcgatgttgaatcgtttaacgtgtcacatgatgc

SEQ ID NO: 43 - DNA, 35 bp, Staphylococcus aureus
  source 1..35: mol_type = other DNA
tgactaaccgaagaagtcgtgtcagatacatttcg

SEQ ID NO: 44 - DNA, 35 bp, Staphylococcus aureus
  source 1..35: mol_type = other DNA
tgaatcgaaatgtatctgacacgacttcttcggtt

SEQ ID NO: 45 - DNA, 70 bp, Staphylococcus aureus
  source 1..70: mol_type = other DNA
gtggtctatagtgcatccctatgcagtcctaatgctgggatttctgccttagtgacaagttttctgaagc

SEQ ID NO: 46 - DNA, 35 bp, Escherichia coli
  source 1..35: mol_type = other DNA
gcattaggactgcatagggatgcactatagaccac

SEQ ID NO: 47 - DNA, 35 bp, Escherichia coli
  source 1..35: mol_type = other DNA
agagccttcttaatggcagactctacgaaagacac

SEQ ID NO: 48 - DNA, 30 bp, Escherichia coli
  source 1..30: mol_type = other DNA
atgcccttgcgttaggcattgagtatctcc

SEQ ID NO: 49 - DNA, 30 bp, Escherichia coli
  source 1..30: mol_type = other DNA
gctccaacatgaagatggctatcgtgtcac

SEQ ID NO: 50 - DNA, 30 bp, Escherichia coli
  source 1..30: mol_type = other DNA
ctgtttgagggtggatagcagtacctgagc

SEQ ID NO: 51 - DNA, 30 bp, Escherichia coli
  source 1..30: mol_type = other DNA
aaatcggtaggtgactctatgccgcagtag

SEQ ID NO: 52 - DNA, 20 bp, Escherichia coli
  source 1..20: mol_type = other DNA
agtccatgcagttggattcc

SEQ ID NO: 53 - DNA, 20 bp, Escherichia coli
  source 1..20: mol_type = other DNA
ttcaagtgcgtttcgtgtgg

SEQ ID NO: 54 - DNA, 21 bp, Escherichia coli
  source 1..21: mol_type = other DNA
atggaaaccgcggtagcgtac

SEQ ID NO: 55 - DNA, 22 bp, Escherichia coli
  source 1..22: mol_type = other DNA
cttttctactgaaccgcgatcc

SEQ ID NO: 56 - DNA, 40 bp, Escherichia coli
  source 1..40: mol_type = other DNA
tacgctaccgcggtttccatggatcctttctcctggtacc

SEQ ID NO: 57 - DNA, 40 bp, Escherichia coli
  source 1..40: mol_type = other DNA
atcgcggttcagtagaaaaggttttggcggatgagagaag

SEQ ID NO: 58 - DNA, 92 bp, Escherichia coli
  source 1..92: mol_type = other DNA
ggagataggggcctttacgattattactttaagatttaactctaagaaggagatatacatatggaaaccgcggtagcgtactataaagatgg

SEQ ID NO: 59 - DNA, 91 bp, Escherichia coli
  source 1..91: mol_type = other DNA
tcgtaaaggcccctatctccctatagtgagtcgtattaatttagggaccttgagtttagataagctgtcaaacatgagcagatcctctacg

SEQ ID NO: 60 - DNA, 20 bp, Escherichia coli
  source 1..20: mol_type = other DNA
gctgcattattagcatgagc

SEQ ID NO: 61 - DNA, 20 bp, Escherichia coli
  source 1..20: mol_type = other DNA
cgaaagcaaaggcaaacagg

SEQ ID NO: 62 - DNA, 20 bp, Escherichia coli
  source 1..20: mol_type = other DNA
tcaccaagagccaatgatcc

SEQ ID NO: 63 - DNA, 20 bp, Escherichia coli
  source 1..20: mol_type = other DNA
cggtgaagtatgatgactgg

SEQ ID NO: 64 - DNA, 20 bp, Escherichia coli
  source 1..20: mol_type = other DNA
gcatcttatctgacacaagg

SEQ ID NO: 65 - DNA, 34 bp, Escherichia coli
  source 1..34: mol_type = other DNA
tccacggatggactctcaaggaggtacaaggtgc

SEQ ID NO: 66 - DNA, 35 bp, Escherichia coli; identical to SEQ ID NO: 14
  source 1..35: mol_type = other DNA

SEQ ID NO: 67 - DNA, 35 bp, Escherichia coli; identical to SEQ ID NO: 15
  source 1..35: mol_type = other DNA

SEQ ID NO: 68 - DNA, 35 bp, Escherichia coli; identical to SEQ ID NO: 16
  source 1..35: mol_type = other DNA

SEQ ID NO: 69 - DNA, 35 bp, Escherichia coli; identical to SEQ ID NO: 17
  source 1..35: mol_type = other DNA

SEQ ID NO: 70 - DNA, 43 bp, Escherichia coli; identical to SEQ ID NO: 18
  source 1..43: mol_type = other DNA

SEQ ID NO: 71 - DNA, 82 bp, Escherichia coli
  source 1..82: mol_type = other DNA
cttagccagaataatcaagtcgttacacgacactaagtgataaactcaaggtccctaaattaatacgactcactatagggag

SEQ ID NO: 72 - DNA, 64 bp, Escherichia coli
  source 1..64: mol_type = other DNA
atgatagcaccttgtacctccttgagagtccatccgtggactactgaaccgcgatccccgtcag